European Patent Application EP 4 556 554 A1, published May 21, 2025. Title: BIFIDOBACTERIUM LONGUM SUBSP. INFANTIS FOR ALLEVIATING PARKINSON'S DISEASE AND USE THEREOF. Applicant: WECARE PROBIOTICS CO., LTD. The sequence listing filed with the application follows.

SEQUENCE LISTING (2 sequences)

SEQ ID NO: 1 - DNA, 1376 bp, synthetic construct
  source 1..1376: mol_type = other DNA
acaaggggttaggccaccggcttcgggtgctgcccactttcatgacttgacgggcggtgtgtacaaggcccgggaacgcattcaccgcgacgttgctgattcgcgattactagcgactccgccttcacgcagtcgagttgcagactgcgatccgaactgagaccggttttcagggatccgctccgcgtcgccgcgtcgcatcccgttgtaccggccattgtagcatgcgtgaagccctggacgtaaggggcatgatgatctgacgtcatccccaccttcctccgagttaaccccggcggtcccccgtgagttcccggcacaatccgctggcaacacggggcgagggttgcgctcgttgcgggacttaacccaacatctcacgacacgagctgacgacgaccatgcaccacctgtgaacccgccccgaagggaaaccccatctctgggatcgtcgggaacatgtcaagcccaggtaaggttcttcgcgttgcatcgaattaatccgcatgctccgccgcttgtgcgggcccccgtcaatttctttgagttttagccttgcggccgtactccccaggcgggatgcttaacgcgttagctccgacacggaacccgtggaacgggccccacatccagcatccaccgtttacggcgtggactaccagggtatctaatcctgttcgctccccacgctttcgctcctcagcgtcagtaacggcccagagacctgccttcgccattggtgttcttcccgatatctacacattccaccgttacaccgggaattccagtctcccctaccgcactcaagcccgcccgtacccggcgcggatccaccgttaagcgatggactttcacaccggacgcgacgaaccgcctacgagccctttacgcccaataattccggataacgcttgcaccctacgtattaccgcggctgctggcacgtagttagccggtgcttattcaacgggtaaactcactcacgcttgctccccgataaaagaggtttacaacccgaaggcctccatccctcacgcggcgtcgctgcatcaggcttgcgcccattgtgcaatattccccactgctgcctcccgtaggagtctgggccgtatctcagtcccaatgtggccggtcgccctctcaggccggctacccgtcgaagccacggtgggccgttaccccgccgtcaagctgataggacgcgaccccatcccataccgcgaaagctttcccagaagaccatgcgatcaactggaacatccggcattaccacccgtttccaggagctattccggtgtatggggcaggtcggtcacgcattactcacccgttcgccactctcaccaccaagcaagcttgatggatcccgttcgact

SEQ ID NO: 2 - DNA, 946 bp, synthetic construct
  source 1..946: mol_type = other DNA
cgcacagcgaaggtcaggccttcctccatggcgatgggctgaatcagctcaacggtgaaggtggcgtggtcgccgggctgaaccatctcgacgccttccggcagctcgatgacgccggtgacgtcggtggtgcggaagtagaactgcggacggtagttggagaagaacggcgagtgacggccgccctcgtccttggtcagcacgtagacttcgccctcgaacttggtgtgcggggtgacggagcctggcttggccacgacctgaccgcgctcgacatcctcacggccgaggccacgcagcagcagaccggtgttatcgccagcctcgcaggcgtccatggtcttgtggaaggtctcgatggaggtgacggtggtggtctgggtcggacggatgccgacgatctcgaccggggtgttgacggccagctggccacgctcgacacgaccggtgacgacggtaccacggccggagatggtgaagacgtcctcgatcggcatcaggaacggcttgtccaggtcgtgaaccggggtcgggatgtagtcatcgacggcggccatgaggtccttgacggactggacccacttctcgtggtccggagcgtcgtcgtgcagggcgccgtaggcggaggtgtggatgaccgggcagtcgcgatcgaagccgttctcgtcgaggaggtcacggacctcttcttcgacgagctcgatgagctcttcatcgtcgaccatgtcgcacttgttgagggcgacaggatcttcgggacgccgacctgacgggcgagcagcacgtgctcgcgggtctgggccatcgggccgtcggtggcggccacaacagggatggccgccatccatctgggcagcaccggtgatcatgttcttcacgaagtcggcgtggcccgggcagtcgacgtgagcgtagtgacgcttctcggtctggtactcgatgtggg